European Patent Application EP 4 552 647 A1, published May 14, 2025. Title: Anti-CCR8 antibody and use thereof. Applicant: Sichuan Swiftbio Biotechnology Co., Ltd. Application WO PCT/CN2023/105817, filed July 5, 2023. The sequence listing filed with the application follows.

SEQUENCE LISTING (60 sequences)

SEQ ID NO: 1 - protein, 115 aa, synthetic construct
QVQLVESGAEVKKPGSSVKVSCKASGYTFTDYEIHWVRQAPGQGLEWMGAIKPETGGTAYAQKFQGRVTLTSDKSTSTAYMELSSLRSEDTAVYYCTRRRYFDVWGQGTLVTVSS

SEQ ID NO: 2 - protein, 112 aa, synthetic construct
DAVMTQTPLSLSVTPGQPASISCRSSQSLEHSDGITYLHWYLQKPGQSPQLLIYRVSNRFSGVPDRFSGSGSGTDFTLKISRVEAEDVGVYYCLQVTHVPFTFGQGTKVEIK

SEQ ID NO: 3 - protein, 7 aa, synthetic construct
GYTFTDY

SEQ ID NO: 4 - protein, 6 aa, synthetic construct
KPETGG

SEQ ID NO: 5 - protein, 6 aa, synthetic construct
RRYFDV

SEQ ID NO: 6 - protein, 10 aa, synthetic construct
GYTFTDYEIH

SEQ ID NO: 7 - protein, 10 aa, synthetic construct
AIKPETGGTA

SEQ ID NO: 8 - protein, 5 aa, synthetic construct
DYEIH

SEQ ID NO: 9 - protein, 17 aa, synthetic construct
AIKPETGGTAYAQKFQG

SEQ ID NO: 10 - protein, 8 aa, synthetic construct
GYTFTDYE

SEQ ID NO: 11 - protein, 8 aa, synthetic construct
IKPETGGT

SEQ ID NO: 12 - protein, 8 aa, synthetic construct
TRRRYFDV

SEQ ID NO: 13 - protein, 16 aa, synthetic construct
RSSQSLEHSDGITYLH

SEQ ID NO: 14 - protein, 7 aa, synthetic construct
RVSNRFS

SEQ ID NO: 15 - protein, 9 aa, synthetic construct
LQVTHVPFT

SEQ ID NO: 16 - protein, 11 aa, synthetic construct
QSLEHSDGITY

SEQ ID NO: 17 - skipped

SEQ ID NO: 18 - protein, 115 aa, synthetic construct
QVQLVESGAEVKKPGSSVKVSCKASGYTFTDYEMHWVRQAPGQGLEWMGAFDPKTGGTAYAQKFQGRVTLTADKSTSTAYMELSSLRSEDTAVYYCARRRFFDVWGQGTLVTVSS

SEQ ID NO: 19 - protein, 112 aa, synthetic construct
DAVMTQTPLSLSVTPGQPASISCRSSQSLEHSNGNTYLHWYLQKPGQSPQLLIYRVSNRFSGVPDRFSGSGSGTDFTLKISRVEAEDVGVYYCLQVTHVPFTFGQGTKVEIK

SEQ ID NO: 20 - protein, 7 aa, synthetic construct
GYTFTDY

SEQ ID NO: 21 - protein, 6 aa, synthetic construct
DPKTGG

SEQ ID NO: 22 - protein, 6 aa, synthetic construct
RRFFDV

SEQ ID NO: 23 - protein, 10 aa, synthetic construct
GYTFTDYEMH

SEQ ID NO: 24 - protein, 10 aa, synthetic construct
AFDPKTGGTA

SEQ ID NO: 25 - protein, 5 aa, synthetic construct
DYEMH

SEQ ID NO: 26 - protein, 17 aa, synthetic construct
AFDPKTGGTAYAQKFQG

SEQ ID NO: 27 - protein, 8 aa, synthetic construct
GYTFTDYE

SEQ ID NO: 28 - protein, 8 aa, synthetic construct
FDPKTGGT

SEQ ID NO: 29 - protein, 8 aa, synthetic construct
ARRRFFDV

SEQ ID NO: 30 - protein, 16 aa, synthetic construct
RSSQSLEHSNGNTYLH

SEQ ID NO: 31 - protein, 7 aa, synthetic construct
RVSNRFS

SEQ ID NO: 32 - protein, 9 aa, synthetic construct
LQVTHVPFT

SEQ ID NO: 33 - protein, 11 aa, synthetic construct
QSLEHSNGNTY

SEQ ID NO: 34 - skipped

SEQ ID NO: 35 - protein, 123 aa, synthetic construct
EVQLVESGGGLVQPGESLRLSCAASGFTFNAYAMNWVRQAPGQGLEWVARIRTKSNNYATYYADSVKGRFTISRDDSKNTLYLEMNSLRAEDTAVYYCVRHKKVREGYAMDYWGQGTLVTVSS

SEQ ID NO: 36 - protein, 111 aa, synthetic construct
DIVLTQSPASLVLSLGQRATISCRASKSVSTSGYTYMHWYQQKPGQPPKLLIYLASNLESGVPARFSGSGSGTDFTLNIHPVEEEDAATYYCQHSRELPFTFGSGTKLEIK

SEQ ID NO: 37 - protein, 7 aa, synthetic construct
GFTFNAY

SEQ ID NO: 38 - protein, 8 aa, synthetic construct
RTKSNNYA

SEQ ID NO: 39 - protein, 12 aa, synthetic construct
HKKVREGYAMDY

SEQ ID NO: 40 - protein, 10 aa, synthetic construct
GFTFNAYAMN

SEQ ID NO: 41 - protein, 12 aa, synthetic construct
RIRTKSNNYATY

SEQ ID NO: 42 - protein, 5 aa, synthetic construct
AYAMN

SEQ ID NO: 43 - protein, 19 aa, synthetic construct
RIRTKSNNYATYYADSVKG

SEQ ID NO: 44 - protein, 8 aa, synthetic construct
GFTFNAYA

SEQ ID NO: 45 - protein, 10 aa, synthetic construct
IRTKSNNYAT

SEQ ID NO: 46 - protein, 14 aa, synthetic construct
VRHKKVREGYAMDY

SEQ ID NO: 47 - protein, 15 aa, synthetic construct
RASKSVSTSGYTYMH

SEQ ID NO: 48 - protein, 7 aa, synthetic construct
LASNLES

SEQ ID NO: 49 - protein, 9 aa, synthetic construct
QHSRELPFT

SEQ ID NO: 50 - protein, 10 aa, synthetic construct
KSVSTSGYTY

SEQ ID NO: 51 - skipped

SEQ ID NO: 52 - protein, 107 aa, synthetic construct [sequence omitted]

SEQ ID NO: 53 - protein, 330 aa, synthetic construct [sequence omitted]

SEQ ID NO: 54 - protein, 330 aa, synthetic construct
ASTKGPSVFPLAPSSKSTSGGTAALGCLVKDYFPEPVTVSWNSGALTSGVHTFPAVLQSSGLYSLSSVVTVPSSSLGTQTYICNVNHKPSNTKVDKKVEPKSCDKTHTCPPCPAPELVGGPSVFLLPPKPKDTLMISRTPEVTCVVVDVSHEDPEVKFNWYVDGVEVHNAKTKPPEEQYNSTLRVVSVLTVLHQDWLNGKEYKCKVSNKALPAPIEKTISKAKGQPREPQVYTLPPSREEMTKNQVSLTCLVKGFYPSDIAVEWESNGQPENNYKTTPLVLDSDGSFFLYSKLTVDKSRWQQGNVFSCSVMHEALHNHYTQKSLSLSPGK

SEQ ID NO: 55 - protein, 123 aa, synthetic construct
EVQLVESGGGLVRPKGSLKFSCAASGFTFNAYAMNWVRQAPGKGLEWVARIRTKSNNYATYYADSVKDRFTISRDDSENMLYLQMNNLKTEDTAIYYCVRHKKVREGYAMDYWGQGTSVTVSS

SEQ ID NO: 56 - protein, 111 aa, synthetic construct; identical to SEQ ID NO: 36

SEQ ID NO: 57 - protein, 115 aa, synthetic construct
QVQLQQSGAELVRPGASVTLSCKASGYTFTDYEMHWVKQTPVHGLEWIGAFDPKTGGTAYNQKFKGKAILTADKSSSTAYMELRSLTSEDSAVYYCARRRFFDVWGAGTTVTVSS

SEQ ID NO: 58 - protein, 112 aa, synthetic construct
DAVMTQTPLSLPVSLGDQASISCRSSQSLEHSNGNTYLHWYLQKPGQSPQLLIYRVSNRFSGVLDRFSGSGSGTDFTLKISRVEAEDLGVYFCLQVTHVPFTFGTGTKLEIK

SEQ ID NO: 59 - protein, 115 aa, synthetic construct
QVQLQQSGAELVRPGASVTLSCKASGYTFTDYEIHWVKMTPAHGLEWIGAIKPETGGTAYNQKFKGKAILTSDKSSSAAYMDLRSLTSEDSAVYYCTRRRYFDVWGAGTTVTVSS

SEQ ID NO: 60 - protein, 112 aa, synthetic construct
DAVMTQTPLSLLVNLGDQASISRRFSQSLEHSDGITYLHWYLQKPGQSPQLLIYRVSIRFCGVVDRFSGSGSGTDFTLKISRVEGEDLGVYFCLQVPQVPFTFGAGTKLEIK